European Patent Specification EP 3 354 726 B1, published October 30, 2024. Title: Process for the modification of a glycoprotein using a glycosyltransferase that is or is derived from a -(1,4)-N-acetylgalactosaminyltransferase. Applicant: SynAffix B.V. The sequence listing filed with the application follows.

SEQUENCE LISTING (92 sequences)

SEQ ID NO: 1 - protein, 402 aa, Artificial
  Bos Taurus GalT Y289L mutant
MKFREPLLGGSAAMPGASLQRACRLLVAVCALHLGVTLVYYLAGRDLRRLPQLVGVHPPLQGSSHGAAAIGQPSGELRLRGVAPPPPLQNSSKPRSRAPSNLDAYSHPGPGPGPGSNLTSAPVPSTTTRSLTACPEESPLLVGPMLIEFNIPVDLKLIEQQNPKVKLGGRYTPMDCISPHKVAIIILFRNRQEHLKYWLYYLHPMVQRQQLDYGIYVINQAGESMFNRAKLLNVGFKEALKDYDYNCFVFSDVDLIPMNDHNTYRCFSQPRHISVAMDKFGFSLPYVQLFGGVSALSKQQFLSINGFPNNYWGWGGEDDDIYNRLAFRGMSVSRPNAVIGKCRMIRHSRDKKNEPNPQRFDRIAHTKETMLSDGLNSLTYMVLEVQRYPLYTKITVDIGTPS

SEQ ID NO: 2 - protein, 383 aa, Caenorhabditis elegans
MAFRHLAVARLKSLLVLCAVLLLVHAMIYKIPSLYENLTIGSSTLIADVDAMEAVLGNTASTSDDLLDTWNSTFSPISEVNQTSFMEDIRPILFPDNQTLQFCNQTPPHLVGPIRVFLDEPDFKTLEKIYPDTHAGGHGMPKDCVARHRVAIIVPYRDREAHLRIMLHNLHSLLAKQQLDYAIFIVEQVANQTFNRGKLMNVGYDVASRLYPWQCFIFHDVDLLPEDDRNLYTCPIQPRHMSVAIDKFNYKLPYSAIFGGISALTKDHLKKINGFSNDFWGWGGEDDDLATRTSMAGLKVSRYPTQIARYKMIKHSTEATNPVNKCRYKIMGQTKRRWTRDGLSNLKYKLVNLELKPLYTRAVVDLLEKDCRRELRRDFPTCF

SEQ ID NO: 3 - protein, 383 aa, Ascaris suum
MNSKLKLVIVLTLCVAIIHFLLSDCPISPDYSFWSPAFIISAPKTLTTLQPFSQSTSTNDLAVSALESVEFSMLDNSSILHASDNWTNDELVMRAQNENLQLCPMTPPALVGPIKVWMDAPSFAELERLYPFLEPGGHGMPTACRARHRVAIVVPYRDRESHLRTFLHNLHSLLTKQQLDYAIFVVEQTANETFNRAKLMNVGYAEAIRLYDWRCFIFHDVDLLPEDDRNLYSCPDEPRHMSVAVDKFNYKLPYGSIFGGISALTREQFEGINGFSNDYWGWGGEDDDLSTRVTLAGYKISRYPAEIARYKMIKHNSEKKNPVNRCRYKLMSATKSRWRNDGLSSLSYDLISLGRLPLYTHIKVDLLEKQSRRYLRTHGFPTC

SEQ ID NO: 4 - protein, 421 aa, Trichoplusia ni
MGGRATRALRLLLLLVLALAAVEYLFGSILDASPLRTYLYTPLYNATQPTLRNVERLAANWPKKIPSNYIEDSEEYSIKNISLSNHTTRASVVHPPSSITETASKLDKNMTIQDGAFAMISPTPLLITKLMDSIKSYVTTEDGVKKAEAVVTLPLCDSMPPDLGPITLNKTELELEWVEKKFPEVEWGGRYSPPNCTARHRVAIIVPYRDRQQHLAIFLNHMHPFLMKQQIEYGIFIVEQEGNKDFNRAKLMNVGFVESQKLVAEGWQCFVFHDIDLLPLDTRNLYSCPRQPRHMSASIDKLHFKLPYEDIFGGVSAMTLEQFTRVNGFSNKYWGWGGEDDDMSYRLKKINYHIARYKMSIARYAMLDHKKSTPNPKRYQLLSQTSKTFQKDGLSTLEYELVQVVQYHLYTHILVNIDERS

SEQ ID NO: 5 - protein, 403 aa, Drosophila melanogaster
MYLFTKANLIRFLAGAICLLLVLNFVGFRSDGGSATSLSKLSIRRVHKYAHIYGNASSDGAGGSEASRLPASPLALSKDRERDQELNGGPNSTIRTVIATANFTSIPQDLTRFLLGTKKFLPPRQKSTSALLANCTDPDPRDGGPITPNTTLESLDVIEAELGPLLRPGGAFEPENCNAQHHVAIVVPFRDRYAHLLLFLRNIHPFLMKQRIAYRIFIVEQTNGKPFNRAAMMNIGYLEALKLYQWDCFIFHDVDLLPLDDRNLYNCPRQPRHMSVAIDTLNFRLPYRSIFGGVSAMTREHFQAVNGFSNSFFGWGGEDDDMSNRLKHANLFISRYPVNIARYKMLKHQKEKANPKRYENLQNGMSKIEQDGINSIKYSIYSIKQFPTFTWYLAELKNSERKS

SEQ ID NO: 6 - protein, 354 aa, Artificial
  CeGalNAcT(30-383)
KIPSLYENLTIGSSTLIADVDAMEAVLGNTASTSDDLLDTWNSTFSPISEVNQTSFMEDIRPILFPDNQTLQFCNQTPPHLVGPIRVFLDEPDFKTLEKIYPDTHAGGHGMPKDCVARHRVAIIVPYRDREAHLRIMLHNLHSLLAKQQLDYAIFIVEQVANQTFNRGKLMNVGYDVASRLYPWQCFIFHDVDLLPEDDRNLYTCPIQPRHMSVAIDKFNYKLPYSAIFGGISALTKDHLKKINGFSNDFWGWGGEDDDLATRTSMAGLKVSRYPTQIARYKMIKHSTEATNPVNKCRYKIMGQTKRRWTRDGLSNLKYKLVNLELKPLYTRAVVDLLEKDCRRELRRDFPTCF

SEQ ID NO: 7 - protein, 354 aa, Artificial
  AsGalNAcT (30-383)
DYSFWSPAFIISAPKTLTTLQPFSQSTSTNDLAVSALESVEFSMLDNSSILHASDNWTNDELVMRAQNENLQLCPMTPPALVGPIKVWMDAPSFAELERLYPFLEPGGHGMPTACRARHRVAIVVPYRDRESHLRTFLHNLHSLLTKQQLDYAIFVVEQTANETFNRAKLMNVGYAEAIRLYDWRCFIFHDVDLLPEDDRNLYSCPDEPRHMSVAVDKFNYKLPYGSIFGGISALTREQFEGINGFSNDYWGWGGEDDDLSTRVTLAGYKISRYPAEIARYKMIKHNSEKKNPVNRCRYKLMSATKSRWRNDGLSSLSYDLISLGRLPLYTHIKVDLLEKQSRRYLRTHGFPTC

SEQ ID NO: 8 - protein, 389 aa, Artificial
  TnGalNAcT(33-421)
SPLRTYLYTPLYNATQPTLRNVERLAANWPKKIPSNYIEDSEEYSIKNISLSNHTTRASVVHPPSSITETASKLDKNMTIQDGAFAMISPTPLLITKLMDSIKSYVTTEDGVKKAEAVVTLPLCDSMPPDLGPITLNKTELELEWVEKKFPEVEWGGRYSPPNCTARHRVAIIVPYRDRQQHLAIFLNHMHPFLMKQQIEYGIFIVEQEGNKDFNRAKLMNVGFVESQKLVAEGWQCFVFHDIDLLPLDTRNLYSCPRQPRHMSASIDKLHFKLPYEDIFGGVSAMTLEQFTRVNGFSNKYWGWGGEDDDMSYRLKKINYHIARYKMSIARYAMLDHKKSTPNPKRYQLLSQTSKTFQKDGLSTLEYELVQVVQYHLYTHILVNIDERS

SEQ ID NO: 9 - protein, 357 aa, Artificial
  DmGalNAcT (47-403)
HKYAHIYGNASSDGAGGSEASRLPASPLALSKDRERDQELNGGPNSTIRTVIATANFTSIPQDLTRFLLGTKKFLPPRQKSTSALLANCTDPDPRDGGPITPNTTLESLDVIEAELGPLLRPGGAFEPENCNAQHHVAIVVPFRDRYAHLLLFLRNIHPFLMKQRIAYRIFIVEQTNGKPFNRAAMMNIGYLEALKLYQWDCFIFHDVDLLPLDDRNLYNCPRQPRHMSVAIDTLNFRLPYRSIFGGVSAMTREHFQAVNGFSNSFFGWGGEDDDMSNRLKHANLFISRYPVNIARYKMLKHQKEKANPKRYENLQNGMSKIEQDGINSIKYSIYSIKQFPTFTWYLAELKNSERKS

SEQ ID NO: 10 - protein, 354 aa, Artificial
  CeGalNacT(30-383; I257L)
KIPSLYENLTIGSSTLIADVDAMEAVLGNTASTSDDLLDTWNSTFSPISEVNQTSFMEDIRPILFPDNQTLQFCNQTPPHLVGPIRVFLDEPDFKTLEKIYPDTHAGGHGMPKDCVARHRVAIIVPYRDREAHLRIMLHNLHSLLAKQQLDYAIFIVEQVANQTFNRGKLMNVGYDVASRLYPWQCFIFHDVDLLPEDDRNLYTCPIQPRHMSVAIDKFNYKLPYSALFGGISALTKDHLKKINGFSNDFWGWGGEDDDLATRTSMAGLKVSRYPTQIARYKMIKHSTEATNPVNKCRYKIMGQTKRRWTRDGLSNLKYKLVNLELKPLYTRAVVDLLEKDCRRELRRDFPTCF

SEQ ID NO: 11 - protein, 354 aa, Artificial
  CeGalNAcT(30-383; I257M)
KIPSLYENLTIGSSTLIADVDAMEAVLGNTASTSDDLLDTWNSTFSPISEVNQTSFMEDIRPILFPDNQTLQFCNQTPPHLVGPIRVFLDEPDFKTLEKIYPDTHAGGHGMPKDCVARHRVAIIVPYRDREAHLRIMLHNLHSLLAKQQLDYAIFIVEQVANQTFNRGKLMNVGYDVASRLYPWQCFIFHDVDLLPEDDRNLYTCPIQPRHMSVAIDKFNYKLPYSAMFGGISALTKDHLKKINGFSNDFWGWGGEDDDLATRTSMAGLKVSRYPTQIARYKMIKHSTEATNPVNKCRYKIMGQTKRRWTRDGLSNLKYKLVNLELKPLYTRAVVDLLEKDCRRELRRDFPTCF

SEQ ID NO: 12 - protein, 354 aa, Artificial
  CeGalNacT(30-383; I257A)
KIPSLYENLTIGSSTLIADVDAMEAVLGNTASTSDDLLDTWNSTFSPISEVNQTSFMEDIRPILFPDNQTLQFCNQTPPHLVGPIRVFLDEPDFKTLEKIYPDTHAGGHGMPKDCVARHRVAIIVPYRDREAHLRIMLHNLHSLLAKQQLDYAIFIVEQVANQTFNRGKLMNVGYDVASRLYPWQCFIFHDVDLLPEDDRNLYTCPIQPRHMSVAIDKFNYKLPYSAAFGGISALTKDHLKKINGFSNDFWGWGGEDDDLATRTSMAGLKVSRYPTQIARYKMIKHSTEATNPVNKCRYKIMGQTKRRWTRDGLSNLKYKLVNLELKPLYTRAVVDLLEKDCRRELRRDFPTCF

SEQ ID NO: 13 - protein, 354 aa, Artificial
  CeGalNacT(30-383; M312H)
KIPSLYENLTIGSSTLIADVDAMEAVLGNTASTSDDLLDTWNSTFSPISEVNQTSFMEDIRPILFPDNQTLQFCNQTPPHLVGPIRVFLDEPDFKTLEKIYPDTHAGGHGMPKDCVARHRVAIIVPYRDREAHLRIMLHNLHSLLAKQQLDYAIFIVEQVANQTFNRGKLMNVGYDVASRLYPWQCFIFHDVDLLPEDDRNLYTCPIQPRHMSVAIDKFNYKLPYSAIFGGISALTKDHLKKINGFSNDFWGWGGEDDDLATRTSMAGLKVSRYPTQIARYKHIKHSTEATNPVNKCRYKIMGQTKRRWTRDGLSNLKYKLVNLELKPLYTRAVVDLLEKDCRRELRRDFPTCF

SEQ ID NO: 14 - protein, 360 aa, Artificial
  CeGalNAcT(30-383)-His
KIPSLYENLTIGSSTLIADVDAMEAVLGNTASTSDDLLDTWNSTFSPISEVNQTSFMEDIRPILFPDNQTLQFCNQTPPHLVGPIRVFLDEPDFKTLEKIYPDTHAGGHGMPKDCVARHRVAIIVPYRDREAHLRIMLHNLHSLLAKQQLDYAIFIVEQVANQTFNRGKLMNVGYDVASRLYPWQCFIFHDVDLLPEDDRNLYTCPIQPRHMSVAIDKFNYKLPYSAIFGGISALTKDHLKKINGFSNDFWGWGGEDDDLATRTSMAGLKVSRYPTQIARYKMIKHSTEATNPVNKCRYKIMGQTKRRWTRDGLSNLKYKLVNLELKPLYTRAVVDLLEKDCRRELRRDFPTCFHHHHHH

SEQ ID NO: 15 - protein, 383 aa, Caenorhabditis remanei
MALRHLAVAKLKTFFVLCAALLLVHTMIYKAPSLYENFSIGSSTLIADVDAMEAVLGNTASTSYDLLDTWNSTFSPISEVNQTSFLEDVRPILFTDNQTKPFCNQTPPHLVGPIRVFLDEPDFATLEKIYPDVHTGGHGIPDECIARHRVAVIVPYRDREAHLRIMLHNLHSLLAKQQLDYAIIVVEQIVNQTFNRGKLMNVGYDVASRLYPWQCFIFHDVDLLPEDDRNLYTCPIQPRHMSVAIDKFDYKLPYSTIFGGISALTQEHVKKINGFSNDFWGWGGEDDDLATRTSMAGLKVSRYPAQIARYKMIKHSTEATNPVNKCRYKIMGQTKRRWTRDGLSSLKYKLVKLDLKPLYTRAVVDLLEKDCRRELRKDFPTCF

SEQ ID NO: 16 - protein, 384 aa, Caenorhabditis briggsae
MAFRHLASAKLKTFFVLCAALLLVHAMIYKVPSLYENFSIGSSTLIADVDAMEAVLGNTASTSDDPFDVWNSTFSPISEVNQTAFMEDIRPILFGDANETRPHCNQTPPHLVGPIRVFLDEPDFATLEKIYPETHPGGHGIPTECVARHRVAIIVPYRDREAHLRIMLHNLHSLLAKQQLDYAIFVVEQVANQTFNRGKLMNVGYDVASRLYPWQCFIFHDVDLLPEDDRNLYTCPIQPRHMSVAIDKFHYKLPYSAIFGGISALTQEHVKAINGFSNDFWGWGGEDDDLATRTSQAGLKVSRYPAQIARYKMIKHSTEATNPVNKCRYKIMGQTKRRWKTDGLSSLKYKLVKLELKPLYTRAVVDLLEKECRRELRRDFPTCF

SEQ ID NO: 17 - protein, 464 aa, Wuchereria bancrofti
MPAAGRFVIILLIFGAAAHIFLGGGLSFISDYHIWRPVVESSRQEIVLVHNIDNNSDQNAEKIISNNETKFHLTSATPIDNLVSIHSNFYELFINGLRFGKLTTVYPIINQSINNGSTTDKSTETYAESVYFLKTDGNIHSNTLLSTITDAQSTRQLFGNETLSACNVIPSFQMMHQNLSLVNCPVTPPGLVGPIKVWYDEPTFEEIERLNPNLEAGGHGKPENCLSRHRVAVIVPYRDREAHLRILLHNLHSLLTKQQLDYGIFVIEQHENETFNRAKLMNVGYVEALKLYDWQCFVFHDVDLLAEDDRNIYSCPDQPRHMSVAVNKFKYKLPYGSIFGGVSAIRTEQFATLNGFSNSYWGWGGEDDDLSMRVTSAGYKIMRYPSEIARYQMVQHKSEMKNPINRCRYDLLAKTKVRQQTDGISSLKYECYDLQFFTLFTHIKVKLFEQESKAQLREEGFKRC

SEQ ID NO: 18 - protein, 291 aa, Loa loa
MERQNLSLVDCPIIPPGLVGPIKVWYDEPTFEEIERLNPYLELGGHGKPGSCLSRHRVAIIVPYRDREAHLRILLHNLHSLLTKQQLDYAIFVIEQHENETFNRAKLMNVGYTEAMKLYDWQCFIFHDVDLLAEDDRNIYSCPDQPRHMSVAINKFKYRLPYGSIFGGVSAIRTEQFLKMNGFSNSYWGWGGEDDDLSIRVTSLGYKIMRYPLEIARYQMVKHESETKNPINRCRYDLLAKTKVRQQMDGISSLKYECYDLHFLPLFTHIKVKLFEQESKAQLREEGFKKC

SEQ ID NO: 19 - protein, 296 aa, Cerapachys biroi
MPIRNLAGNGGTARELPVANTTSNATIPRCPLIPPNLVGPVAVSKSPPPLSEMERSFVEVKAGGKGRPADCVARHRVAIIIPFRDRPQHLQTLLYNLHPILLRQQIDYQIFVIEQEGTGTFNRAMLMNVGYVEALKERIFDCFIFHDVDLLPEDDRNLYTCPEQPRHMSVAVDKFKYRLPYADLFGGVSAMSREHFQLVNGFSNVFWGWGGEDDDMANRIKAHGLHISRYPANVARYKMLTHKKEKANPKRYEFLKTGKKRFSTDGLANLQYELCDKRKPKLYTWLLVRLTPPQPS

SEQ ID NO: 20 - protein, 422 aa, Zootermopsis nevadensis
MRCRCLSAWSRITQHVPRQPCLHIHSHLCKVVIVLAVLIALQFLLTTIFEARQIEPLFTVNFTYSGRRSRWGLISHSRGLLSPSHNSSFNGSMRVSVERTLSPVENISGETKNLSFLHTHENAVRNASSLVLNISLPSDLNPTTSPSLTVPFTGKSLCPPIPPNLNGPIKVLKDSPSLEELEKMFPLLEPGGHYHPEECQARDRVAIIVPYRDRAEHLSTFLLNLHPLLQRQQLDYGMFVIEQGGDGPFNRAMLMNVGFVEALKLYSYDCFIFHDVDLLPEDDRNLYTCPEQPRHMSVAVDVLKYKLPYQAIFGGVSAMTKTQFQKVNGFSNLFWGWGGEDDDMSNRVRHHGYHISRYPANIARYKMLAHRKQHANPKRYEFLNTGRKRFKTDGLSNLQYDRKELNLGKLYTRVLVELATPS

SEQ ID NO: 21 - protein, 295 aa, Camponotus floridanus
MPTRNLVGGGTARELPVANATNNTTMPRCPLIPPNLVGPMVVSKSPPPLSEMERSFVEVNAGGRGRPADCVARHRVAIIIPFRDRPQHLQTLLYNLHPILLRQQIEYQIFVIEQEGTGAFNRAMLMNVGYVEALKERTFDCFIFHDVDLLPEDDRNLYTCPEQPRHMSVAVDKFKYRLPYTDLFGGVSAMSREHFQLVNGFSNVFWGWGGEDDDMANRIKAHGLHISRYPANVARYKMLTHKKEKANPKRYEFLKTGKKRFSTDGLANLQYELSDKRKPKLYTWLLVRLTPPQPS

SEQ ID NO: 22 - protein, 310 aa, Crassostrea gigas
MDRGCKPMRVCSSSPSDLVGSLATYKEAPSYKEMIKIYPLVRPGGLYTPPDCIARERVAIIIPFRDREEHLRILLHNLHPMLQRQQLDYGIYVVEQENGTQFNRAMLMNIGYAESIKLYNYTCFIFHDVDLIPENDRIMYDCRDSPRHLSSAVDKFKYKLPYPQLFGGVTAIKRAHFEKVNGHSNKFFGWGGEDDDMFRRLVNNGFKISRYQASLSKYKMIKHLHDAGNKANKRRHHLIKTGKGRYRRDGINNLHYKKLGIEYQYLHTRILVSINETKVMTVSLLYMYSSTTVYIIVNIYTIYCKSRNIR

SEQ ID NO: 23 - protein, 338 aa, Danaus plexippus
MAKKLLTQGTESVTNYTHTTNSSNKNPAKETFNMTKPNLSDDTSTPLLITKIMESIKNLVTTEEDFRDEPSLPLCDEMPPDLGPISVNKTEIELDWVEKRYPEVRSGGIYSSSNCTARHRVAIIVPYRDRQQHLAIFLNHMHPFLMKQQIEYGIYIIEQEGTSEFNRAKLMNVGFVESQRQRSWQCFIFHDIDLLPLDSRNMYSCPKQPRHMSASIDKLNFRLPYEDIFGGVSAMTLEQFTKVNGFSNKYWGWGGEDDDMFYRLKKMNYHIARYKMSIARYAMLDHKKSAPNPKRYQLLSQTSKTFQKDGLSTLEYEVIKVTANHLYTHILVNIDERS

SEQ ID NO: 24 - protein, 941 aa, Artificial
  HuGalNAcT (57-998)
RYGSWRELAKALASRNIPAVDPHLQFYHPQRLSLEDHDIDQGVSSNSSYLKWNKPVPWLSEFRGRANLHVFEDWCGSSIQQLRRNLHFPLYPHIRTTLRKLAVSPKWTNYGLRIFGYLHPFTDGKIQFAIAADDNAEFWLSLDDQVSGLQLLASVGKTGKEWTAPGEFGKFRSQISKPVSLSASHRYYFEVLHKQNEEGTDHVEVAWRRNDPGAKFTIIDSLSLSLFTNETFLQMDEVGHIPQTAASHVDSSNALPRDEQPPADMLRPDPRDTLYRVPLIPKSHLRHVLPDCPYKPSYLVDGLPLQRYQGLRFVHLSFVYPNDYTRLSHMETHNKCFYQENAYYQDRFSFQEYIKIDQPEKQGLEQPGFEENLLEESQYGEVAEETPASNNQNARMLEGRQTPASTLEQDATDYRLRSLRKLLAQPREGLLAPFSKRNSTASFPGRTSHIPVQQPEKRKQKPSPEPSQDSPHSDKWPPGHPVKNLPQMRGPRPRPAGDSPRKTQWLNQVESYIAEQRRGDRMRPQAPGRGWHGEEEVVAAAGQEGQVEGEEEGEEEEEEEDMSEVFEYVPVFDPVVNWDQTFSARNLDFQALRTDWIDLSCNTSGNLLLPEQEALEVTRVFLKKLNQRSRGRYQLQRIVNVEKRQDQLRGGRYLLELELLEQGQRVVRLSEYVSARGWQGIDPAGGEEVEARNLQGLVWDPHNRRRQVLNTRAQEPKLCWPQGFSWSHRAVVHFVVPVKNQARWVQQFIKDMENLFQVTGDPHFNIVITDYSSEDMDVEMALKRSKLRSYQYVKLSGNFERSAGLQAGIDLVKDPHSIIFLCDLHIHFPAGVIDAIRKHCVEGKMAFAPMVMRLHCGATPQWPEGYWEVNGFGLLGIYKSDLDRIGGMNTKEFRDRWGGEDWELLDRILQGLDVERLSLRNFFHHFHSKRGMWSRRQMKTL

SEQ ID NO: 25 - protein, 389 aa, Artificial
  TnGalNAcT(33-421; W336F)
SPLRTYLYTPLYNATQPTLRNVERLAANWPKKIPSNYIEDSEEYSIKNISLSNHTTRASVVHPPSSITETASKLDKNMTIQDGAFAMISPTPLLITKLMDSIKSYVTTEDGVKKAEAVVTLPLCDSMPPDLGPITLNKTELELEWVEKKFPEVEWGGRYSPPNCTARHRVAIIVPYRDRQQHLAIFLNHMHPFLMKQQIEYGIFIVEQEGNKDFNRAKLMNVGFVESQKLVAEGWQCFVFHDIDLLPLDTRNLYSCPRQPRHMSASIDKLHFKLPYEDIFGGVSAMTLEQFTRVNGFSNKYWGFGGEDDDMSYRLKKINYHIARYKMSIARYAMLDHKKSTPNPKRYQLLSQTSKTFQKDGLSTLEYELVQVVQYHLYTHILVNIDERS

SEQ ID NO: 26 - protein, 389 aa, Artificial
  TnGalNAcT(33-421; W336H)
SPLRTYLYTPLYNATQPTLRNVERLAANWPKKIPSNYIEDSEEYSIKNISLSNHTTRASVVHPPSSITETASKLDKNMTIQDGAFAMISPTPLLITKLMDSIKSYVTTEDGVKKAEAVVTLPLCDSMPPDLGPITLNKTELELEWVEKKFPEVEWGGRYSPPNCTARHRVAIIVPYRDRQQHLAIFLNHMHPFLMKQQIEYGIFIVEQEGNKDFNRAKLMNVGFVESQKLVAEGWQCFVFHDIDLLPLDTRNLYSCPRQPRHMSASIDKLHFKLPYEDIFGGVSAMTLEQFTRVNGFSNKYWGHGGEDDDMSYRLKKINYHIARYKMSIARYAMLDHKKSTPNPKRYQLLSQTSKTFQKDGLSTLEYELVQVVQYHLYTHILVNIDERS

SEQ ID NO: 27 - protein, 389 aa, Artificial
  TnGalNAcT(33-421; W336V)
SPLRTYLYTPLYNATQPTLRNVERLAANWPKKIPSNYIEDSEEYSIKNISLSNHTTRASVVHPPSSITETASKLDKNMTIQDGAFAMISPTPLLITKLMDSIKSYVTTEDGVKKAEAVVTLPLCDSMPPDLGPITLNKTELELEWVEKKFPEVEWGGRYSPPNCTARHRVAIIVPYRDRQQHLAIFLNHMHPFLMKQQIEYGIFIVEQEGNKDFNRAKLMNVGFVESQKLVAEGWQCFVFHDIDLLPLDTRNLYSCPRQPRHMSASIDKLHFKLPYEDIFGGVSAMTLEQFTRVNGFSNKYWGVGGEDDDMSYRLKKINYHIARYKMSIARYAMLDHKKSTPNPKRYQLLSQTSKTFQKDGLSTLEYELVQVVQYHLYTHILVNIDERS

SEQ ID NO: 28 - protein, 389 aa, Artificial
  TnGalNAcT(33-421; E339A)
SPLRTYLYTPLYNATQPTLRNVERLAANWPKKIPSNYIEDSEEYSIKNISLSNHTTRASVVHPPSSITETASKLDKNMTIQDGAFAMISPTPLLITKLMDSIKSYVTTEDGVKKAEAVVTLPLCDSMPPDLGPITLNKTELELEWVEKKFPEVEWGGRYSPPNCTARHRVAIIVPYRDRQQHLAIFLNHMHPFLMKQQIEYGIFIVEQEGNKDFNRAKLMNVGFVESQKLVAEGWQCFVFHDIDLLPLDTRNLYSCPRQPRHMSASIDKLHFKLPYEDIFGGVSAMTLEQFTRVNGFSNKYWGWGGADDDMSYRLKKINYHIARYKMSIARYAMLDHKKSTPNPKRYQLLSQTSKTFQKDGLSTLEYELVQVVQYHLYTHILVNIDERS

SEQ ID NO: 29 - protein, 389 aa, Artificial
  TnGalNAcT(33-421; E339G)
SPLRTYLYTPLYNATQPTLRNVERLAANWPKKIPSNYIEDSEEYSIKNISLSNHTTRASVVHPPSSITETASKLDKNMTIQDGAFAMISPTPLLITKLMDSIKSYVTTEDGVKKAEAVVTLPLCDSMPPDLGPITLNKTELELEWVEKKFPEVEWGGRYSPPNCTARHRVAIIVPYRDRQQHLAIFLNHMHPFLMKQQIEYGIFIVEQEGNKDFNRAKLMNVGFVESQKLVAEGWQCFVFHDIDLLPLDTRNLYSCPRQPRHMSASIDKLHFKLPYEDIFGGVSAMTLEQFTRVNGFSNKYWGWGGGDDDMSYRLKKINYHIARYKMSIARYAMLDHKKSTPNPKRYQLLSQTSKTFQKDGLSTLEYELVQVVQYHLYTHILVNIDERS

SEQ ID NO: 30 - protein, 389 aa, Artificial
  TnGalNAcT(33-421; E339D)
SPLRTYLYTPLYNATQPTLRNVERLAANWPKKIPSNYIEDSEEYSIKNISLSNHTTRASVVHPPSSITETASKLDKNMTIQDGAFAMISPTPLLITKLMDSIKSYVTTEDGVKKAEAVVTLPLCDSMPPDLGPITLNKTELELEWVEKKFPEVEWGGRYSPPNCTARHRVAIIVPYRDRQQHLAIFLNHMHPFLMKQQIEYGIFIVEQEGNKDFNRAKLMNVGFVESQKLVAEGWQCFVFHDIDLLPLDTRNLYSCPRQPRHMSASIDKLHFKLPYEDIFGGVSAMTLEQFTRVNGFSNKYWGWGGDDDDMSYRLKKINYHIARYKMSIARYAMLDHKKSTPNPKRYQLLSQTSKTFQKDGLSTLEYELVQVVQYHLYTHILVNIDERS

SEQ ID NO: 31 - protein, 389 aa, Artificial
  TnGalNAcT(33-421; E339S)
SPLRTYLYTPLYNATQPTLRNVERLAANWPKKIPSNYIEDSEEYSIKNISLSNHTTRASVVHPPSSITETASKLDKNMTIQDGAFAMISPTPLLITKLMDSIKSYVTTEDGVKKAEAVVTLPLCDSMPPDLGPITLNKTELELEWVEKKFPEVEWGGRYSPPNCTARHRVAIIVPYRDRQQHLAIFLNHMHPFLMKQQIEYGIFIVEQEGNKDFNRAKLMNVGFVESQKLVAEGWQCFVFHDIDLLPLDTRNLYSCPRQPRHMSASIDKLHFKLPYEDIFGGVSAMTLEQFTRVNGFSNKYWGWGGSDDDMSYRLKKINYHIARYKMSIARYAMLDHKKSTPNPKRYQLLSQTSKTFQKDGLSTLEYELVQVVQYHLYTHILVNIDERS

SEQ ID NO: 32 - protein, 389 aa, Artificial
  TnGalNAcT(33-421; W336H,E339A)
SPLRTYLYTPLYNATQPTLRNVERLAANWPKKIPSNYIEDSEEYSIKNISLSNHTTRASVVHPPSSITETASKLDKNMTIQDGAFAMISPTPLLITKLMDSIKSYVTTEDGVKKAEAVVTLPLCDSMPPDLGPITLNKTELELEWVEKKFPEVEWGGRYSPPNCTARHRVAIIVPYRDRQQHLAIFLNHMHPFLMKQQIEYGIFIVEQEGNKDFNRAKLMNVGFVESQKLVAEGWQCFVFHDIDLLPLDTRNLYSCPRQPRHMSASIDKLHFKLPYEDIFGGVSAMTLEQFTRVNGFSNKYWGHGGADDDMSYRLKKINYHIARYKMSIARYAMLDHKKSTPNPKRYQLLSQTSKTFQKDGLSTLEYELVQVVQYHLYTHILVNIDERS

SEQ ID NO: 33 - protein, 389 aa, Artificial
  TnGalNAcT(33-421; W336H,E339D)
SPLRTYLYTPLYNATQPTLRNVERLAANWPKKIPSNYIEDSEEYSIKNISLSNHTTRASVVHPPSSITETASKLDKNMTIQDGAFAMISPTPLLITKLMDSIKSYVTTEDGVKKAEAVVTLPLCDSMPPDLGPITLNKTELELEWVEKKFPEVEWGGRYSPPNCTARHRVAIIVPYRDRQQHLAIFLNHMHPFLMKQQIEYGIFIVEQEGNKDFNRAKLMNVGFVESQKLVAEGWQCFVFHDIDLLPLDTRNLYSCPRQPRHMSASIDKLHFKLPYEDIFGGVSAMTLEQFTRVNGFSNKYWGHGGDDDDMSYRLKKINYHIARYKMSIARYAMLDHKKSTPNPKRYQLLSQTSKTFQKDGLSTLEYELVQVVQYHLYTHILVNIDERS

SEQ ID NO: 34 - protein, 389 aa, Artificial
  TnGalNAcT(33-421; W336H,E339S)
SPLRTYLYTPLYNATQPTLRNVERLAANWPKKIPSNYIEDSEEYSIKNISLSNHTTRASVVHPPSSITETASKLDKNMTIQDGAFAMISPTPLLITKLMDSIKSYVTTEDGVKKAEAVVTLPLCDSMPPDLGPITLNKTELELEWVEKKFPEVEWGGRYSPPNCTARHRVAIIVPYRDRQQHLAIFLNHMHPFLMKQQIEYGIFIVEQEGNKDFNRAKLMNVGFVESQKLVAEGWQCFVFHDIDLLPLDTRNLYSCPRQPRHMSASIDKLHFKLPYEDIFGGVSAMTLEQFTRVNGFSNKYWGHGGSDDDMSYRLKKINYHIARYKMSIARYAMLDHKKSTPNPKRYQLLSQTSKTFQKDGLSTLEYELVQVVQYHLYTHILVNIDERS

SEQ ID NO: 35 - protein, 389 aa, Artificial
  TnGalNAcT(33-421; I311Y)
SPLRTYLYTPLYNATQPTLRNVERLAANWPKKIPSNYIEDSEEYSIKNISLSNHTTRASVVHPPSSITETASKLDKNMTIQDGAFAMISPTPLLITKLMDSIKSYVTTEDGVKKAEAVVTLPLCDSMPPDLGPITLNKTELELEWVEKKFPEVEWGGRYSPPNCTARHRVAIIVPYRDRQQHLAIFLNHMHPFLMKQQIEYGIFIVEQEGNKDFNRAKLMNVGFVESQKLVAEGWQCFVFHDIDLLPLDTRNLYSCPRQPRHMSASIDKLHFKLPYEDYFGGVSAMTLEQFTRVNGFSNKYWGWGGEDDDMSYRLKKINYHIARYKMSIARYAMLDHKKSTPNPKRYQLLSQTSKTFQKDGLSTLEYELVQVVQYHLYTHILVNIDERS

SEQ ID NO: 36 - protein, 389 aa, Artificial
  TnGalNAcT(33-421; I311Y,W336F)
SPLRTYLYTPLYNATQPTLRNVERLAANWPKKIPSNYIEDSEEYSIKNISLSNHTTRASVVHPPSSITETASKLDKNMTIQDGAFAMISPTPLLITKLMDSIKSYVTTEDGVKKAEAVVTLPLCDSMPPDLGPITLNKTELELEWVEKKFPEVEWGGRYSPPNCTARHRVAIIVPYRDRQQHLAIFLNHMHPFLMKQQIEYGIFIVEQEGNKDFNRAKLMNVGFVESQKLVAEGWQCFVFHDIDLLPLDTRNLYSCPRQPRHMSASIDKLHFKLPYEDYFGGVSAMTLEQFTRVNGFSNKYWGFGGEDDDMSYRLKKINYHIARYKMSIARYAMLDHKKSTPNPKRYQLLSQTSKTFQKDGLSTLEYELVQVVQYHLYTHILVNIDERS

SEQ ID NO: 37 - protein, 389 aa, Artificial
  TnGalNAcT(33-421; I311Y,W336H)
SPLRTYLYTPLYNATQPTLRNVERLAANWPKKIPSNYIEDSEEYSIKNISLSNHTTRASVVHPPSSITETASKLDKNMTIQDGAFAMISPTPLLITKLMDSIKSYVTTEDGVKKAEAVVTLPLCDSMPPDLGPITLNKTELELEWVEKKFPEVEWGGRYSPPNCTARHRVAIIVPYRDRQQHLAIFLNHMHPFLMKQQIEYGIFIVEQEGNKDFNRAKLMNVGFVESQKLVAEGWQCFVFHDIDLLPLDTRNLYSCPRQPRHMSASIDKLHFKLPYEDYFGGVSAMTLEQFTRVNGFSNKYWGHGGEDDDMSYRLKKINYHIARYKMSIARYAMLDHKKSTPNPKRYQLLSQTSKTFQKDGLSTLEYELVQVVQYHLYTHILVNIDERS

SEQ ID NO: 38 - protein, 389 aa, Artificial
  TnGalNAcT(33-421; I311Y,W336V)
SPLRTYLYTPLYNATQPTLRNVERLAANWPKKIPSNYIEDSEEYSIKNISLSNHTTRASVVHPPSSITETASKLDKNMTIQDGAFAMISPTPLLITKLMDSIKSYVTTEDGVKKAEAVVTLPLCDSMPPDLGPITLNKTELELEWVEKKFPEVEWGGRYSPPNCTARHRVAIIVPYRDRQQHLAIFLNHMHPFLMKQQIEYGIFIVEQEGNKDFNRAKLMNVGFVESQKLVAEGWQCFVFHDIDLLPLDTRNLYSCPRQPRHMSASIDKLHFKLPYEDYFGGVSAMTLEQFTRVNGFSNKYWGVGGEDDDMSYRLKKINYHIARYKMSIARYAMLDHKKSTPNPKRYQLLSQTSKTFQKDGLSTLEYELVQVVQYHLYTHILVNIDERS

SEQ ID NO: 39 - protein, 389 aa, Artificial
  TnGalNAcT(33-421; I311Y,E339A)
SPLRTYLYTPLYNATQPTLRNVERLAANWPKKIPSNYIEDSEEYSIKNISLSNHTTRASVVHPPSSITETASKLDKNMTIQDGAFAMISPTPLLITKLMDSIKSYVTTEDGVKKAEAVVTLPLCDSMPPDLGPITLNKTELELEWVEKKFPEVEWGGRYSPPNCTARHRVAIIVPYRDRQQHLAIFLNHMHPFLMKQQIEYGIFIVEQEGNKDFNRAKLMNVGFVESQKLVAEGWQCFVFHDIDLLPLDTRNLYSCPRQPRHMSASIDKLHFKLPYEDYFGGVSAMTLEQFTRVNGFSNKYWGWGGADDDMSYRLKKINYHIARYKMSIARYAMLDHKKSTPNPKRYQLLSQTSKTFQKDGLSTLEYELVQVVQYHLYTHILVNIDERS

SEQ ID NO: 40 - protein, 389 aa, Artificial
  TnGalNAcT(33-421; I311Y,E339G)
SPLRTYLYTPLYNATQPTLRNVERLAANWPKKIPSNYIEDSEEYSIKNISLSNHTTRASVVHPPSSITETASKLDKNMTIQDGAFAMISPTPLLITKLMDSIKSYVTTEDGVKKAEAVVTLPLCDSMPPDLGPITLNKTELELEWVEKKFPEVEWGGRYSPPNCTARHRVAIIVPYRDRQQHLAIFLNHMHPFLMKQQIEYGIFIVEQEGNKDFNRAKLMNVGFVESQKLVAEGWQCFVFHDIDLLPLDTRNLYSCPRQPRHMSASIDKLHFKLPYEDYFGGVSAMTLEQFTRVNGFSNKYWGWGGGDDDMSYRLKKINYHIARYKMSIARYAMLDHKKSTPNPKRYQLLSQTSKTFQKDGLSTLEYELVQVVQYHLYTHILVNIDERS

SEQ ID NO: 41 - protein, 389 aa, Artificial
  TnGalNAcT(33-421; I311Y,E339D)
SPLRTYLYTPLYNATQPTLRNVERLAANWPKKIPSNYIEDSEEYSIKNISLSNHTTRASVVHPPSSITETASKLDKNMTIQDGAFAMISPTPLLITKLMDSIKSYVTTEDGVKKAEAVVTLPLCDSMPPDLGPITLNKTELELEWVEKKFPEVEWGGRYSPPNCTARHRVAIIVPYRDRQQHLAIFLNHMHPFLMKQQIEYGIFIVEQEGNKDFNRAKLMNVGFVESQKLVAEGWQCFVFHDIDLLPLDTRNLYSCPRQPRHMSASIDKLHFKLPYEDYFGGVSAMTLEQFTRVNGFSNKYWGWGGDDDDMSYRLKKINYHIARYKMSIARYAMLDHKKSTPNPKRYQLLSQTSKTFQKDGLSTLEYELVQVVQYHLYTHILVNIDERS

SEQ ID NO: 42 - protein, 389 aa, Artificial
  TnGalNAcT(33-421; I311Y,E339S)
SPLRTYLYTPLYNATQPTLRNVERLAANWPKKIPSNYIEDSEEYSIKNISLSNHTTRASVVHPPSSITETASKLDKNMTIQDGAFAMISPTPLLITKLMDSIKSYVTTEDGVKKAEAVVTLPLCDSMPPDLGPITLNKTELELEWVEKKFPEVEWGGRYSPPNCTARHRVAIIVPYRDRQQHLAIFLNHMHPFLMKQQIEYGIFIVEQEGNKDFNRAKLMNVGFVESQKLVAEGWQCFVFHDIDLLPLDTRNLYSCPRQPRHMSASIDKLHFKLPYEDYFGGVSAMTLEQFTRVNGFSNKYWGWGGSDDDMSYRLKKINYHIARYKMSIARYAMLDHKKSTPNPKRYQLLSQTSKTFQKDGLSTLEYELVQVVQYHLYTHILVNIDERS

SEQ ID NO: 43 - protein, 389 aa, Artificial
  TnGalNAcT(33-421; I311Y,W336H,E339A)
SPLRTYLYTPLYNATQPTLRNVERLAANWPKKIPSNYIEDSEEYSIKNISLSNHTTRASVVHPPSSITETASKLDKNMTIQDGAFAMISPTPLLITKLMDSIKSYVTTEDGVKKAEAVVTLPLCDSMPPDLGPITLNKTELELEWVEKKFPEVEWGGRYSPPNCTARHRVAIIVPYRDRQQHLAIFLNHMHPFLMKQQIEYGIFIVEQEGNKDFNRAKLMNVGFVESQKLVAEGWQCFVFHDIDLLPLDTRNLYSCPRQPRHMSASIDKLHFKLPYEDYFGGVSAMTLEQFTRVNGFSNKYWGHGGADDDMSYRLKKINYHIARYKMSIARYAMLDHKKSTPNPKRYQLLSQTSKTFQKDGLSTLEYELVQVVQYHLYTHILVNIDERS

SEQ ID NO: 44 - protein, 389 aa, Artificial
  TnGalNAcT(33-421; I311Y,W336H,E339D)
SPLRTYLYTPLYNATQPTLRNVERLAANWPKKIPSNYIEDSEEYSIKNISLSNHTTRASVVHPPSSITETASKLDKNMTIQDGAFAMISPTPLLITKLMDSIKSYVTTEDGVKKAEAVVTLPLCDSMPPDLGPITLNKTELELEWVEKKFPEVEWGGRYSPPNCTARHRVAIIVPYRDRQQHLAIFLNHMHPFLMKQQIEYGIFIVEQEGNKDFNRAKLMNVGFVESQKLVAEGWQCFVFHDIDLLPLDTRNLYSCPRQPRHMSASIDKLHFKLPYEDYFGGVSAMTLEQFTRVNGFSNKYWGHGGDDDDMSYRLKKINYHIARYKMSIARYAMLDHKKSTPNPKRYQLLSQTSKTFQKDGLSTLEYELVQVVQYHLYTHILVNIDERS

SEQ ID NO: 45 - protein, 389 aa, Artificial
  TnGalNAcT(33-421; I311Y,W336H,E339S)
SPLRTYLYTPLYNATQPTLRNVERLAANWPKKIPSNYIEDSEEYSIKNISLSNHTTRASVVHPPSSITETASKLDKNMTIQDGAFAMISPTPLLITKLMDSIKSYVTTEDGVKKAEAVVTLPLCDSMPPDLGPITLNKTELELEWVEKKFPEVEWGGRYSPPNCTARHRVAIIVPYRDRQQHLAIFLNHMHPFLMKQQIEYGIFIVEQEGNKDFNRAKLMNVGFVESQKLVAEGWQCFVFHDIDLLPLDTRNLYSCPRQPRHMSASIDKLHFKLPYEDYFGGVSAMTLEQFTRVNGFSNKYWGHGGSDDDMSYRLKKINYHIARYKMSIARYAMLDHKKSTPNPKRYQLLSQTSKTFQKDGLSTLEYELVQVVQYHLYTHILVNIDERS

SEQ ID NO: 46 - protein, 354 aa, Artificial
  AsGalNAcT(30-383; W282H)
DYSFWSPAFIISAPKTLTTLQPFSQSTSTNDLAVSALESVEFSMLDNSSILHASDNWTNDELVMRAQNENLQLCPMTPPALVGPIKVWMDAPSFAELERLYPFLEPGGHGMPTACRARHRVAIVVPYRDRESHLRTFLHNLHSLLTKQQLDYAIFVVEQTANETFNRAKLMNVGYAEAIRLYDWRCFIFHDVDLLPEDDRNLYSCPDEPRHMSVAVDKFNYKLPYGSIFGGISALTREQFEGINGFSNDYWGHGGEDDDLSTRVTLAGYKISRYPAEIARYKMIKHNSEKKNPVNRCRYKLMSATKSRWRNDGLSSLSYDLISLGRLPLYTHIKVDLLEKQSRRYLRTHGFPTC

SEQ ID NO: 47 - protein, 354 aa, Artificial
  AsGalNAcT(30-383; E285D)
DYSFWSPAFIISAPKTLTTLQPFSQSTSTNDLAVSALESVEFSMLDNSSILHASDNWTNDELVMRAQNENLQLCPMTPPALVGPIKVWMDAPSFAELERLYPFLEPGGHGMPTACRARHRVAIVVPYRDRESHLRTFLHNLHSLLTKQQLDYAIFVVEQTANETFNRAKLMNVGYAEAIRLYDWRCFIFHDVDLLPEDDRNLYSCPDEPRHMSVAVDKFNYKLPYGSIFGGISALTREQFEGINGFSNDYWGWGGDDDDLSTRVTLAGYKISRYPAEIARYKMIKHNSEKKNPVNRCRYKLMSATKSRWRNDGLSSLSYDLISLGRLPLYTHIKVDLLEKQSRRYLRTHGFPTC

SEQ ID NO: 48 - protein, 354 aa, Artificial
  AsGalNAcT(30-383; I257Y)
DYSFWSPAFIISAPKTLTTLQPFSQSTSTNDLAVSALESVEFSMLDNSSILHASDNWTNDELVMRAQNENLQLCPMTPPALVGPIKVWMDAPSFAELERLYPFLEPGGHGMPTACRARHRVAIVVPYRDRESHLRTFLHNLHSLLTKQQLDYAIFVVEQTANETFNRAKLMNVGYAEAIRLYDWRCFIFHDVDLLPEDDRNLYSCPDEPRHMSVAVDKFNYKLPYGSYFGGISALTREQFEGINGFSNDYWGWGGEDDDLSTRVTLAGYKISRYPAEIARYKMIKHNSEKKNPVNRCRYKLMSATKSRWRNDGLSSLSYDLISLGRLPLYTHIKVDLLEKQSRRYLRTHGFPTC

SEQ ID NO: 49 - protein, 410 aa, Artificial
  His-TnGalNAcT(33-421)
MGSSHHHHHHSSGLVPRGSHMSPLRTYLYTPLYNATQPTLRNVERLAANWPKKIPSNYIEDSEEYSIKNISLSNHTTRASVVHPPSSITETASKLDKNMTIQDGAFAMISPTPLLITKLMDSIKSYVTTEDGVKKAEAVVTLPLCDSMPPDLGPITLNKTELELEWVEKKFPEVEWGGRYSPPNCTARHRVAIIVPYRDRQQHLAIFLNHMHPFLMKQQIEYGIFIVEQEGNKDFNRAKLMNVGFVESQKLVAEGWQCFVFHDIDLLPLDTRNLYSCPRQPRHMSASIDKLHFKLPYEDIFGGVSAMTLEQFTRVNGFSNKYWGWGGEDDDMSYRLKKINYHIARYKMSIARYAMLDHKKSTPNPKRYQLLSQTSKTFQKDGLSTLEYELVQVVQYHLYTHILVNIDERS

SEQ ID NO: 50 - protein, 410 aa, Artificial
  His-TnGalNAcT(33-421; W336F)
MGSSHHHHHHSSGLVPRGSHMSPLRTYLYTPLYNATQPTLRNVERLAANWPKKIPSNYIEDSEEYSIKNISLSNHTTRASVVHPPSSITETASKLDKNMTIQDGAFAMISPTPLLITKLMDSIKSYVTTEDGVKKAEAVVTLPLCDSMPPDLGPITLNKTELELEWVEKKFPEVEWGGRYSPPNCTARHRVAIIVPYRDRQQHLAIFLNHMHPFLMKQQIEYGIFIVEQEGNKDFNRAKLMNVGFVESQKLVAEGWQCFVFHDIDLLPLDTRNLYSCPRQPRHMSASIDKLHFKLPYEDIFGGVSAMTLEQFTRVNGFSNKYWGFGGEDDDMSYRLKKINYHIARYKMSIARYAMLDHKKSTPNPKRYQLLSQTSKTFQKDGLSTLEYELVQVVQYHLYTHILVNIDERS

SEQ ID NO: 51 - protein, 410 aa, Artificial
  His-TnGalNAcT(33-421; W336H)
MGSSHHHHHHSSGLVPRGSHMSPLRTYLYTPLYNATQPTLRNVERLAANWPKKIPSNYIEDSEEYSIKNISLSNHTTRASVVHPPSSITETASKLDKNMTIQDGAFAMISPTPLLITKLMDSIKSYVTTEDGVKKAEAVVTLPLCDSMPPDLGPITLNKTELELEWVEKKFPEVEWGGRYSPPNCTARHRVAIIVPYRDRQQHLAIFLNHMHPFLMKQQIEYGIFIVEQEGNKDFNRAKLMNVGFVESQKLVAEGWQCFVFHDIDLLPLDTRNLYSCPRQPRHMSASIDKLHFKLPYEDIFGGVSAMTLEQFTRVNGFSNKYWGHGGEDDDMSYRLKKINYHIARYKMSIARYAMLDHKKSTPNPKRYQLLSQTSKTFQKDGLSTLEYELVQVVQYHLYTHILVNIDERS

SEQ ID NO: 52 - protein, 410 aa, Artificial
  His-TnGalNAcT(33-421; W336V)
MGSSHHHHHHSSGLVPRGSHMSPLRTYLYTPLYNATQPTLRNVERLAANWPKKIPSNYIEDSEEYSIKNISLSNHTTRASVVHPPSSITETASKLDKNMTIQDGAFAMISPTPLLITKLMDSIKSYVTTEDGVKKAEAVVTLPLCDSMPPDLGPITLNKTELELEWVEKKFPEVEWGGRYSPPNCTARHRVAIIVPYRDRQQHLAIFLNHMHPFLMKQQIEYGIFIVEQEGNKDFNRAKLMNVGFVESQKLVAEGWQCFVFHDIDLLPLDTRNLYSCPRQPRHMSASIDKLHFKLPYEDIFGGVSAMTLEQFTRVNGFSNKYWGVGGEDDDMSYRLKKINYHIARYKMSIARYAMLDHKKSTPNPKRYQLLSQTSKTFQKDGLSTLEYELVQVVQYHLYTHILVNIDERS

SEQ ID NO: 53 - protein, 410 aa, Artificial
  His-TnGalNAcT(33-421; E339A)
MGSSHHHHHHSSGLVPRGSHMSPLRTYLYTPLYNATQPTLRNVERLAANWPKKIPSNYIEDSEEYSIKNISLSNHTTRASVVHPPSSITETASKLDKNMTIQDGAFAMISPTPLLITKLMDSIKSYVTTEDGVKKAEAVVTLPLCDSMPPDLGPITLNKTELELEWVEKKFPEVEWGGRYSPPNCTARHRVAIIVPYRDRQQHLAIFLNHMHPFLMKQQIEYGIFIVEQEGNKDFNRAKLMNVGFVESQKLVAEGWQCFVFHDIDLLPLDTRNLYSCPRQPRHMSASIDKLHFKLPYEDIFGGVSAMTLEQFTRVNGFSNKYWGWGGADDDMSYRLKKINYHIARYKMSIARYAMLDHKKSTPNPKRYQLLSQTSKTFQKDGLSTLEYELVQVVQYHLYTHILVNIDERS

SEQ ID NO: 54 - protein, 410 aa, Artificial
  His-TnGalNAcT(33-421; E339G)
MGSSHHHHHHSSGLVPRGSHMSPLRTYLYTPLYNATQPTLRNVERLAANWPKKIPSNYIEDSEEYSIKNISLSNHTTRASVVHPPSSITETASKLDKNMTIQDGAFAMISPTPLLITKLMDSIKSYVTTEDGVKKAEAVVTLPLCDSMPPDLGPITLNKTELELEWVEKKFPEVEWGGRYSPPNCTARHRVAIIVPYRDRQQHLAIFLNHMHPFLMKQQIEYGIFIVEQEGNKDFNRAKLMNVGFVESQKLVAEGWQCFVFHDIDLLPLDTRNLYSCPRQPRHMSASIDKLHFKLPYEDIFGGVSAMTLEQFTRVNGFSNKYWGWGGGDDDMSYRLKKINYHIARYKMSIARYAMLDHKKSTPNPKRYQLLSQTSKTFQKDGLSTLEYELVQVVQYHLYTHILVNIDERS

SEQ ID NO: 55 - protein, 410 aa, Artificial
  His-TnGalNAcT(33-421; E339D)
MGSSHHHHHHSSGLVPRGSHMSPLRTYLYTPLYNATQPTLRNVERLAANWPKKIPSNYIEDSEEYSIKNISLSNHTTRASVVHPPSSITETASKLDKNMTIQDGAFAMISPTPLLITKLMDSIKSYVTTEDGVKKAEAVVTLPLCDSMPPDLGPITLNKTELELEWVEKKFPEVEWGGRYSPPNCTARHRVAIIVPYRDRQQHLAIFLNHMHPFLMKQQIEYGIFIVEQEGNKDFNRAKLMNVGFVESQKLVAEGWQCFVFHDIDLLPLDTRNLYSCPRQPRHMSASIDKLHFKLPYEDIFGGVSAMTLEQFTRVNGFSNKYWGWGGDDDDMSYRLKKINYHIARYKMSIARYAMLDHKKSTPNPKRYQLLSQTSKTFQKDGLSTLEYELVQVVQYHLYTHILVNIDERS

SEQ ID NO: 56 - protein, 410 aa, Artificial
  His-TnGalNAcT(33-421; E339S)
MGSSHHHHHHSSGLVPRGSHMSPLRTYLYTPLYNATQPTLRNVERLAANWPKKIPSNYIEDSEEYSIKNISLSNHTTRASVVHPPSSITETASKLDKNMTIQDGAFAMISPTPLLITKLMDSIKSYVTTEDGVKKAEAVVTLPLCDSMPPDLGPITLNKTELELEWVEKKFPEVEWGGRYSPPNCTARHRVAIIVPYRDRQQHLAIFLNHMHPFLMKQQIEYGIFIVEQEGNKDFNRAKLMNVGFVESQKLVAEGWQCFVFHDIDLLPLDTRNLYSCPRQPRHMSASIDKLHFKLPYEDIFGGVSAMTLEQFTRVNGFSNKYWGWGGSDDDMSYRLKKINYHIARYKMSIARYAMLDHKKSTPNPKRYQLLSQTSKTFQKDGLSTLEYELVQVVQYHLYTHILVNIDERS

SEQ ID NO: 57 - protein, 410 aa, Artificial
  His-TnGalNAcT(33-421; W336H,E339A)
MGSSHHHHHHSSGLVPRGSHMSPLRTYLYTPLYNATQPTLRNVERLAANWPKKIPSNYIEDSEEYSIKNISLSNHTTRASVVHPPSSITETASKLDKNMTIQDGAFAMISPTPLLITKLMDSIKSYVTTEDGVKKAEAVVTLPLCDSMPPDLGPITLNKTELELEWVEKKFPEVEWGGRYSPPNCTARHRVAIIVPYRDRQQHLAIFLNHMHPFLMKQQIEYGIFIVEQEGNKDFNRAKLMNVGFVESQKLVAEGWQCFVFHDIDLLPLDTRNLYSCPRQPRHMSASIDKLHFKLPYEDIFGGVSAMTLEQFTRVNGFSNKYWGHGGADDDMSYRLKKINYHIARYKMSIARYAMLDHKKSTPNPKRYQLLSQTSKTFQKDGLSTLEYELVQVVQYHLYTHILVNIDERS

SEQ ID NO: 58 - protein, 410 aa, Artificial
  His-TnGalNAcT(33-421; W336H,E339D)
MGSSHHHHHHSSGLVPRGSHMSPLRTYLYTPLYNATQPTLRNVERLAANWPKKIPSNYIEDSEEYSIKNISLSNHTTRASVVHPPSSITETASKLDKNMTIQDGAFAMISPTPLLITKLMDSIKSYVTTEDGVKKAEAVVTLPLCDSMPPDLGPITLNKTELELEWVEKKFPEVEWGGRYSPPNCTARHRVAIIVPYRDRQQHLAIFLNHMHPFLMKQQIEYGIFIVEQEGNKDFNRAKLMNVGFVESQKLVAEGWQCFVFHDIDLLPLDTRNLYSCPRQPRHMSASIDKLHFKLPYEDIFGGVSAMTLEQFTRVNGFSNKYWGHGGDDDDMSYRLKKINYHIARYKMSIARYAMLDHKKSTPNPKRYQLLSQTSKTFQKDGLSTLEYELVQVVQYHLYTHILVNIDERS

SEQ ID NO: 59 - protein, 410 aa, Artificial
  His-TnGalNAcT(33-421; W336H,E339S)
MGSSHHHHHHSSGLVPRGSHMSPLRTYLYTPLYNATQPTLRNVERLAANWPKKIPSNYIEDSEEYSIKNISLSNHTTRASVVHPPSSITETASKLDKNMTIQDGAFAMISPTPLLITKLMDSIKSYVTTEDGVKKAEAVVTLPLCDSMPPDLGPITLNKTELELEWVEKKFPEVEWGGRYSPPNCTARHRVAIIVPYRDRQQHLAIFLNHMHPFLMKQQIEYGIFIVEQEGNKDFNRAKLMNVGFVESQKLVAEGWQCFVFHDIDLLPLDTRNLYSCPRQPRHMSASIDKLHFKLPYEDIFGGVSAMTLEQFTRVNGFSNKYWGHGGSDDDMSYRLKKINYHIARYKMSIARYAMLDHKKSTPNPKRYQLLSQTSKTFQKDGLSTLEYELVQVVQYHLYTHILVNIDERS

SEQ ID NO: 60 - protein, 410 aa, Artificial
  His-TnGalNAcT(33-421; I311Y)
MGSSHHHHHHSSGLVPRGSHMSPLRTYLYTPLYNATQPTLRNVERLAANWPKKIPSNYIEDSEEYSIKNISLSNHTTRASVVHPPSSITETASKLDKNMTIQDGAFAMISPTPLLITKLMDSIKSYVTTEDGVKKAEAVVTLPLCDSMPPDLGPITLNKTELELEWVEKKFPEVEWGGRYSPPNCTARHRVAIIVPYRDRQQHLAIFLNHMHPFLMKQQIEYGIFIVEQEGNKDFNRAKLMNVGFVESQKLVAEGWQCFVFHDIDLLPLDTRNLYSCPRQPRHMSASIDKLHFKLPYEDYFGGVSAMTLEQFTRVNGFSNKYWGWGGEDDDMSYRLKKINYHIARYKMSIARYAMLDHKKSTPNPKRYQLLSQTSKTFQKDGLSTLEYELVQVVQYHLYTHILVNIDERS

SEQ ID NO: 61 - protein, 410 aa, Artificial
  His-TnGalNAcT(33-421; I311Y,W336F)
MGSSHHHHHHSSGLVPRGSHMSPLRTYLYTPLYNATQPTLRNVERLAANWPKKIPSNYIEDSEEYSIKNISLSNHTTRASVVHPPSSITETASKLDKNMTIQDGAFAMISPTPLLITKLMDSIKSYVTTEDGVKKAEAVVTLPLCDSMPPDLGPITLNKTELELEWVEKKFPEVEWGGRYSPPNCTARHRVAIIVPYRDRQQHLAIFLNHMHPFLMKQQIEYGIFIVEQEGNKDFNRAKLMNVGFVESQKLVAEGWQCFVFHDIDLLPLDTRNLYSCPRQPRHMSASIDKLHFKLPYEDYFGGVSAMTLEQFTRVNGFSNKYWGFGGEDDDMSYRLKKINYHIARYKMSIARYAMLDHKKSTPNPKRYQLLSQTSKTFQKDGLSTLEYELVQVVQYHLYTHILVNIDERS

SEQ ID NO: 62 - protein, 410 aa, Artificial
  His-TnGalNAcT(33-421; I311Y,W336H)
MGSSHHHHHHSSGLVPRGSHMSPLRTYLYTPLYNATQPTLRNVERLAANWPKKIPSNYIEDSEEYSIKNISLSNHTTRASVVHPPSSITETASKLDKNMTIQDGAFAMISPTPLLITKLMDSIKSYVTTEDGVKKAEAVVTLPLCDSMPPDLGPITLNKTELELEWVEKKFPEVEWGGRYSPPNCTARHRVAIIVPYRDRQQHLAIFLNHMHPFLMKQQIEYGIFIVEQEGNKDFNRAKLMNVGFVESQKLVAEGWQCFVFHDIDLLPLDTRNLYSCPRQPRHMSASIDKLHFKLPYEDYFGGVSAMTLEQFTRVNGFSNKYWGHGGEDDDMSYRLKKINYHIARYKMSIARYAMLDHKKSTPNPKRYQLLSQTSKTFQKDGLSTLEYELVQVVQYHLYTHILVNIDERS

SEQ ID NO: 63 - protein, 409 aa, Artificial
  His-TnGalNAcT(33-421; I311Y,W336V)
GSSHHHHHHSSGLVPRGSHMSPLRTYLYTPLYNATQPTLRNVERLAANWPKKIPSNYIEDSEEYSIKNISLSNHTTRASVVHPPSSITETASKLDKNMTIQDGAFAMISPTPLLITKLMDSIKSYVTTEDGVKKAEAVVTLPLCDSMPPDLGPITLNKTELELEWVEKKFPEVEWGGRYSPPNCTARHRVAIIVPYRDRQQHLAIFLNHMHPFLMKQQIEYGIFIVEQEGNKDFNRAKLMNVGFVESQKLVAEGWQCFVFHDIDLLPLDTRNLYSCPRQPRHMSASIDKLHFKLPYEDYFGGVSAMTLEQFTRVNGFSNKYWGVGGEDDDMSYRLKKINYHIARYKMSIARYAMLDHKKSTPNPKRYQLLSQTSKTFQKDGLSTLEYELVQVVQYHLYTHILVNIDERS

SEQ ID NO: 64 - protein, 410 aa, Artificial
  His-TnGalNAcT(33-421; I311Y,E339A)
MGSSHHHHHHSSGLVPRGSHMSPLRTYLYTPLYNATQPTLRNVERLAANWPKKIPSNYIEDSEEYSIKNISLSNHTTRASVVHPPSSITETASKLDKNMTIQDGAFAMISPTPLLITKLMDSIKSYVTTEDGVKKAEAVVTLPLCDSMPPDLGPITLNKTELELEWVEKKFPEVEWGGRYSPPNCTARHRVAIIVPYRDRQQHLAIFLNHMHPFLMKQQIEYGIFIVEQEGNKDFNRAKLMNVGFVESQKLVAEGWQCFVFHDIDLLPLDTRNLYSCPRQPRHMSASIDKLHFKLPYEDYFGGVSAMTLEQFTRVNGFSNKYWGWGGADDDMSYRLKKINYHIARYKMSIARYAMLDHKKSTPNPKRYQLLSQTSKTFQKDGLSTLEYELVQVVQYHLYTHILVNIDERS

SEQ ID NO: 65 - protein, 410 aa, Artificial
  His-TnGalNAcT(33-421; I311Y,E339G)
MGSSHHHHHHSSGLVPRGSHMSPLRTYLYTPLYNATQPTLRNVERLAANWPKKIPSNYIEDSEEYSIKNISLSNHTTRASVVHPPSSITETASKLDKNMTIQDGAFAMISPTPLLITKLMDSIKSYVTTEDGVKKAEAVVTLPLCDSMPPDLGPITLNKTELELEWVEKKFPEVEWGGRYSPPNCTARHRVAIIVPYRDRQQHLAIFLNHMHPFLMKQQIEYGIFIVEQEGNKDFNRAKLMNVGFVESQKLVAEGWQCFVFHDIDLLPLDTRNLYSCPRQPRHMSASIDKLHFKLPYEDYFGGVSAMTLEQFTRVNGFSNKYWGWGGGDDDMSYRLKKINYHIARYKMSIARYAMLDHKKSTPNPKRYQLLSQTSKTFQKDGLSTLEYELVQVVQYHLYTHILVNIDERS

SEQ ID NO: 66 - protein, 410 aa, Artificial
  His-TnGalNAcT(33-421; I311Y,E339D)
MGSSHHHHHHSSGLVPRGSHMSPLRTYLYTPLYNATQPTLRNVERLAANWPKKIPSNYIEDSEEYSIKNISLSNHTTRASVVHPPSSITETASKLDKNMTIQDGAFAMISPTPLLITKLMDSIKSYVTTEDGVKKAEAVVTLPLCDSMPPDLGPITLNKTELELEWVEKKFPEVEWGGRYSPPNCTARHRVAIIVPYRDRQQHLAIFLNHMHPFLMKQQIEYGIFIVEQEGNKDFNRAKLMNVGFVESQKLVAEGWQCFVFHDIDLLPLDTRNLYSCPRQPRHMSASIDKLHFKLPYEDYFGGVSAMTLEQFTRVNGFSNKYWGWGGDDDDMSYRLKKINYHIARYKMSIARYAMLDHKKSTPNPKRYQLLSQTSKTFQKDGLSTLEYELVQVVQYHLYTHILVNIDERS

SEQ ID NO: 67 - protein, 410 aa, Artificial
  His-TnGalNAcT(33-421; I311Y,E339S)
MGSSHHHHHHSSGLVPRGSHMSPLRTYLYTPLYNATQPTLRNVERLAANWPKKIPSNYIEDSEEYSIKNISLSNHTTRASVVHPPSSITETASKLDKNMTIQDGAFAMISPTPLLITKLMDSIKSYVTTEDGVKKAEAVVTLPLCDSMPPDLGPITLNKTELELEWVEKKFPEVEWGGRYSPPNCTARHRVAIIVPYRDRQQHLAIFLNHMHPFLMKQQIEYGIFIVEQEGNKDFNRAKLMNVGFVESQKLVAEGWQCFVFHDIDLLPLDTRNLYSCPRQPRHMSASIDKLHFKLPYEDYFGGVSAMTLEQFTRVNGFSNKYWGWGGSDDDMSYRLKKINYHIARYKMSIARYAMLDHKKSTPNPKRYQLLSQTSKTFQKDGLSTLEYELVQVVQYHLYTHILVNIDERS

SEQ ID NO: 68 - protein, 410 aa, Artificial
  His-TnGalNAcT(33-421; I311Y,W336H,E339A)
MGSSHHHHHHSSGLVPRGSHMSPLRTYLYTPLYNATQPTLRNVERLAANWPKKIPSNYIEDSEEYSIKNISLSNHTTRASVVHPPSSITETASKLDKNMTIQDGAFAMISPTPLLITKLMDSIKSYVTTEDGVKKAEAVVTLPLCDSMPPDLGPITLNKTELELEWVEKKFPEVEWGGRYSPPNCTARHRVAIIVPYRDRQQHLAIFLNHMHPFLMKQQIEYGIFIVEQEGNKDFNRAKLMNVGFVESQKLVAEGWQCFVFHDIDLLPLDTRNLYSCPRQPRHMSASIDKLHFKLPYEDYFGGVSAMTLEQFTRVNGFSNKYWGHGGADDDMSYRLKKINYHIARYKMSIARYAMLDHKKSTPNPKRYQLLSQTSKTFQKDGLSTLEYELVQVVQYHLYTHILVNIDERS

SEQ ID NO: 69 - protein, 410 aa, Artificial
  His-TnGalNAcT(33-421; I311Y,W336H,E339D)
MGSSHHHHHHSSGLVPRGSHMSPLRTYLYTPLYNATQPTLRNVERLAANWPKKIPSNYIEDSEEYSIKNISLSNHTTRASVVHPPSSITETASKLDKNMTIQDGAFAMISPTPLLITKLMDSIKSYVTTEDGVKKAEAVVTLPLCDSMPPDLGPITLNKTELELEWVEKKFPEVEWGGRYSPPNCTARHRVAIIVPYRDRQQHLAIFLNHMHPFLMKQQIEYGIFIVEQEGNKDFNRAKLMNVGFVESQKLVAEGWQCFVFHDIDLLPLDTRNLYSCPRQPRHMSASIDKLHFKLPYEDYFGGVSAMTLEQFTRVNGFSNKYWGHGGDDDDMSYRLKKINYHIARYKMSIARYAMLDHKKSTPNPKRYQLLSQTSKTFQKDGLSTLEYELVQVVQYHLYTHILVNIDERS

SEQ ID NO: 70 - protein, 410 aa, Artificial
  His-TnGalNAcT(33-421; I311Y,W336H,E339S)
MGSSHHHHHHSSGLVPRGSHMSPLRTYLYTPLYNATQPTLRNVERLAANWPKKIPSNYIEDSEEYSIKNISLSNHTTRASVVHPPSSITETASKLDKNMTIQDGAFAMISPTPLLITKLMDSIKSYVTTEDGVKKAEAVVTLPLCDSMPPDLGPITLNKTELELEWVEKKFPEVEWGGRYSPPNCTARHRVAIIVPYRDRQQHLAIFLNHMHPFLMKQQIEYGIFIVEQEGNKDFNRAKLMNVGFVESQKLVAEGWQCFVFHDIDLLPLDTRNLYSCPRQPRHMSASIDKLHFKLPYEDYFGGVSAMTLEQFTRVNGFSNKYWGHGGSDDDMSYRLKKINYHIARYKMSIARYAMLDHKKSTPNPKRYQLLSQTSKTFQKDGLSTLEYELVQVVQYHLYTHILVNIDERS

SEQ ID NO: 71 - protein, 375 aa, Artificial
  His-AsGalNAcT(30-383)
MGSSHHHHHHSSGLVPRGSHMDYSFWSPAFIISAPKTLTTLQPFSQSTSTNDLAVSALESVEFSMLDNSSILHASDNWTNDELVMRAQNENLQLCPMTPPALVGPIKVWMDAPSFAELERLYPFLEPGGHGMPTACRARHRVAIVVPYRDRESHLRTFLHNLHSLLTKQQLDYAIFVVEQTANETFNRAKLMNVGYAEAIRLYDWRCFIFHDVDLLPEDDRNLYSCPDEPRHMSVAVDKFNYKLPYGSIFGGISALTREQFEGINGFSNDYWGWGGEDDDLSTRVTLAGYKISRYPAEIARYKMIKHNSEKKNPVNRCRYKLMSATKSRWRNDGLSSLSYDLISLGRLPLYTHIKVDLLEKQSRRYLRTHGFPTC

SEQ ID NO: 72 - protein, 375 aa, Artificial
  His-AsGalNAcT(30-383; W282H)
MGSSHHHHHHSSGLVPRGSHMDYSFWSPAFIISAPKTLTTLQPFSQSTSTNDLAVSALESVEFSMLDNSSILHASDNWTNDELVMRAQNENLQLCPMTPPALVGPIKVWMDAPSFAELERLYPFLEPGGHGMPTACRARHRVAIVVPYRDRESHLRTFLHNLHSLLTKQQLDYAIFVVEQTANETFNRAKLMNVGYAEAIRLYDWRCFIFHDVDLLPEDDRNLYSCPDEPRHMSVAVDKFNYKLPYGSIFGGISALTREQFEGINGFSNDYWGHGGEDDDLSTRVTLAGYKISRYPAEIARYKMIKHNSEKKNPVNRCRYKLMSATKSRWRNDGLSSLSYDLISLGRLPLYTHIKVDLLEKQSRRYLRTHGFPTC

SEQ ID NO: 73 - protein, 375 aa, Artificial
  His-AsGalNAcT(30-383; E285D)
MGSSHHHHHHSSGLVPRGSHMDYSFWSPAFIISAPKTLTTLQPFSQSTSTNDLAVSALESVEFSMLDNSSILHASDNWTNDELVMRAQNENLQLCPMTPPALVGPIKVWMDAPSFAELERLYPFLEPGGHGMPTACRARHRVAIVVPYRDRESHLRTFLHNLHSLLTKQQLDYAIFVVEQTANETFNRAKLMNVGYAEAIRLYDWRCFIFHDVDLLPEDDRNLYSCPDEPRHMSVAVDKFNYKLPYGSIFGGISALTREQFEGINGFSNDYWGWGGDDDDLSTRVTLAGYKISRYPAEIARYKMIKHNSEKKNPVNRCRYKLMSATKSRWRNDGLSSLSYDLISLGRLPLYTHIKVDLLEKQSRRYLRTHGFPTC

SEQ ID NO: 74 - protein, 375 aa, Artificial
  His-AsGalNAcT(30-383; I257Y)
MGSSHHHHHHSSGLVPRGSHMDYSFWSPAFIISAPKTLTTLQPFSQSTSTNDLAVSALESVEFSMLDNSSILHASDNWTNDELVMRAQNENLQLCPMTPPALVGPIKVWMDAPSFAELERLYPFLEPGGHGMPTACRARHRVAIVVPYRDRESHLRTFLHNLHSLLTKQQLDYAIFVVEQTANETFNRAKLMNVGYAEAIRLYDWRCFIFHDVDLLPEDDRNLYSCPDEPRHMSVAVDKFNYKLPYGSYFGGISALTREQFEGINGFSNDYWGWGGEDDDLSTRVTLAGYKISRYPAEIARYKMIKHNSEKKNPVNRCRYKLMSATKSRWRNDGLSSLSYDLISLGRLPLYTHIKVDLLEKQSRRYLRTHGFPTC

SEQ ID NO: 75 - DNA, 1173 bp, Artificial
  TnGalNAcT(33-421)
atgtcaccgctgcgtacctacctgtataccccgctgtataatgccacccaaccgaccctgcgtaatgtggaacgtctggctgcgaactggccgaagaaaattccgagcaactatatcgaagattcagaagaatactcgatcaaaaacatcagtctgtccaatcataccacgcgtgcgagtgtggttcacccgccgagctctatcaccgaaacggcctccaaactggacaaaaatatgaccattcaggatggcgcgttcgccatgattagcccgaccccgctgctgatcacgaaactgatggacagcattaaatcttatgtcaccacggaagatggcgtgaagaaagcggaagctgtcgttaccctgccgctgtgtgactccatgccgccagatctgggtccgattaccctgaacaaaacggaactggaactggaatgggttgagaaaaaatttccggaagtcgaatggggcggtcgctatagtccgccgaactgtaccgcacgtcatcgcgtggctattatcgttccgtaccgtgaccgccagcaacacctggcaatctttctgaatcacatgcacccgttcctgatgaaacagcaaattgaatacggcatttttatcgtggaacaggaaggtaataaagatttcaatcgtgcaaaactgatgaacgttggctttgtcgaatctcagaaactggtggctgaaggttggcaatgctttgttttccatgacatcgatctgctgccgctggatacccgcaatctgtatagttgtccgcgccagccgcgtcacatgtcagccagcatcgacaaactgcactttaaactgccgtacgaagatattttcggcggtgtctcagccatgaccctggaacaatttacgcgtgttaacggcttctcgaataaatattggggttggggcggtgaagatgacgatatgagctaccgcctgaagaaaattaactatcatatcgcccgttacaaaatgagcattgcgcgctatgccatgctggaccacaaaaaatctaccccgaatccgaaacgttaccagctgctgagtcaaaccagcaaaacgtttcagaaagatggtctgtctacgctggaatatgaactggtccaagttgtgcagtatcatctgtacacgcatattctggtgaacattgacgaacgctcttga

SEQ ID NO: 76 - DNA, 1233 bp, Artificial
  His-TnGalNAcT(33-421)
atgggcagcagccatcatcatcatcatcacagcagcggcctggtgccgcgcggcagccatatgtcaccgctgcgtacctacctgtataccccgctgtataatgccacccaaccgaccctgcgtaatgtggaacgtctggctgcgaactggccgaagaaaattccgagcaactatatcgaagattcagaagaatactcgatcaaaaacatcagtctgtccaatcataccacgcgtgcgagtgtggttcacccgccgagctctatcaccgaaacggcctccaaactggacaaaaatatgaccattcaggatggcgcgttcgccatgattagcccgaccccgctgctgatcacgaaactgatggacagcattaaatcttatgtcaccacggaagatggcgtgaagaaagcggaagctgtcgttaccctgccgctgtgtgactccatgccgccagatctgggtccgattaccctgaacaaaacggaactggaactggaatgggttgagaaaaaatttccggaagtcgaatggggcggtcgctatagtccgccgaactgtaccgcacgtcatcgcgtggctattatcgttccgtaccgtgaccgccagcaacacctggcaatctttctgaatcacatgcacccgttcctgatgaaacagcaaattgaatacggcatttttatcgtggaacaggaaggtaataaagatttcaatcgtgcaaaactgatgaacgttggctttgtcgaatctcagaaactggtggctgaaggttggcaatgctttgttttccatgacatcgatctgctgccgctggatacccgcaatctgtatagttgtccgcgccagccgcgtcacatgtcagccagcatcgacaaactgcactttaaactgccgtacgaagatattttcggcggtgtctcagccatgaccctggaacaatttacgcgtgttaacggcttctcgaataaatattggggttggggcggtgaagatgacgatatgagctaccgcctgaagaaaattaactatcatatcgcccgttacaaaatgagcattgcgcgctatgccatgctggaccacaaaaaatctaccccgaatccgaaacgttaccagctgctgagtcaaaccagcaaaacgtttcagaaagatggtctgtctacgctggaatatgaactggtccaagttgtgcagtatcatctgtacacgcatattctggtgaacattgacgaacgctcttga

SEQ ID NO: 77 - DNA, 1068 bp, Artificial
  AsGalNAcT(30-383)
atggattactcattctggagcccggcgttcatcatctctgccccgaaaaccctgaccaccctgcaaccgttctctcagtctacctctaccaacgacctggcagtctcagctctggaatcggtggaatttagcatgctggataatagctctattctgcatgcgtctgacaactggaccaatgatgaactggtgatgcgcgcccagaacgaaaatctgcaactgtgtccgatgacgccgccggcgctggttggcccgatcaaagtttggatggatgcgccgagctttgccgaactggaacgtctgtatccgttcctggaaccgggcggtcatggtatgccgaccgcctgtcgtgcacgtcaccgtgttgccattgtggttccgtatcgcgaccgtgaatcccacctgcgcaccttcctgcataacctgcactcactgctgacgaaacagcaactggattacgcaatctttgtcgtggaacagaccgcaaacgaaacgttcaatcgtgctaaactgatgaatgttggctatgcggaagccattcgcctgtacgattggcgttgctttatcttccatgacgtcgatctgctgccggaagatgaccgcaacctgtattcttgtccggacgaaccgcgtcacatgagtgttgcagtcgataaattcaactacaaactgccgtacggttcgattttcggcggtatcagcgctctgacccgcgaacaatttgaaggcattaacggtttcagcaatgattactggggctggggcggtgaagatgacgatctgtcgacccgtgtgacgctggcgggttataaaatcagccgctacccggcagaaatcgctcgttacaaaatgatcaaacataacagtgaaaagaaaaacccggttaatcgctgccgttacaaactgatgtctgccaccaaaagtcgctggcgtaatgacggcctgagttccctgtcctatgatctgatttcactgggtcgcctgccgctgtacacgcacatcaaagttgacctgctggaaaaacaatctcgccgctatctgcgtacccacggcttcccgacctgctga

SEQ ID NO: 78 - DNA, 1128 bp, Artificial
  His-AsGalNAcT(30-383)
atgggcagcagccatcatcatcatcatcacagcagcggcctggtgccgcgcggcagccatatggattactcattctggagcccggcgttcatcatctctgccccgaaaaccctgaccaccctgcaaccgttctctcagtctacctctaccaacgacctggcagtctcagctctggaatcggtggaatttagcatgctggataatagctctattctgcatgcgtctgacaactggaccaatgatgaactggtgatgcgcgcccagaacgaaaatctgcaactgtgtccgatgacgccgccggcgctggttggcccgatcaaagtttggatggatgcgccgagctttgccgaactggaacgtctgtatccgttcctggaaccgggcggtcatggtatgccgaccgcctgtcgtgcacgtcaccgtgttgccattgtggttccgtatcgcgaccgtgaatcccacctgcgcaccttcctgcataacctgcactcactgctgacgaaacagcaactggattacgcaatctttgtcgtggaacagaccgcaaacgaaacgttcaatcgtgctaaactgatgaatgttggctatgcggaagccattcgcctgtacgattggcgttgctttatcttccatgacgtcgatctgctgccggaagatgaccgcaacctgtattcttgtccggacgaaccgcgtcacatgagtgttgcagtcgataaattcaactacaaactgccgtacggttcgattttcggcggtatcagcgctctgacccgcgaacaatttgaaggcattaacggtttcagcaatgattactggggctggggcggtgaagatgacgatctgtcgacccgtgtgacgctggcgggttataaaatcagccgctacccggcagaaatcgctcgttacaaaatgatcaaacataacagtgaaaagaaaaacccggttaatcgctgccgttacaaactgatgtctgccaccaaaagtcgctggcgtaatgacggcctgagttccctgtcctatgatctgatttcactgggtcgcctgccgctgtacacgcacatcaaagttgacctgctggaaaaacaatctcgccgctatctgcgtacccacggcttcccgacctgctga

SEQ ID NO: 79 - DNA, 43 bp, Artificial
  primer sequence W336F, fwd
ctcgaataaatattggggttttggcggtgaagatgacgatatg

SEQ ID NO: 80 - DNA, 43 bp, Artificial
  primer sequence W336F,rev
catatcgtcatcttcaccgccaaaaccccaatatttattcgag

SEQ ID NO: 81 - DNA, 36 bp, Artificial
  primer sequence W336H,fwd
cgaataaatattggggtcacggcggtgaagatgacg

SEQ ID NO: 82 - DNA, 36 bp, Artificial
  primer sequence W336H,rev
cgtcatcttcaccgccgtgaccccaatatttattcg

SEQ ID NO: 83 - DNA, 36 bp, Artificial
  primer sequence W336V,fwd
cgaataaatattggggtgtgggcggtgaagatgacg

SEQ ID NO: 84 - DNA, 36 bp, Artificial
  primer sequence W336V,rev
cgtcatcttcaccgcccacaccccaatatttattcg

SEQ ID NO: 85 - DNA, 31 bp, Artificial
  primer sequence E339A,fwd
gggttggggcggtgcggatgacgatatgagc

SEQ ID NO: 86 - DNA, 31 bp, Artificial
  primer sequence E339A,rev
gctcatatcgtcatccgcaccgccccaaccc

SEQ ID NO: 87 - DNA, 30 bp, Artificial
  primer sequence E339G,fwd
gggttggggcggtggagatgacgatatgag

SEQ ID NO: 88 - DNA, 30 bp, Artificial
  primer sequence E339G,rev
ctcatatcgtcatctccaccgccccaaccc

SEQ ID NO: 89 - DNA, 31 bp, Artificial
  primer sequence E339D,fwd
gggttggggcggtgatgatgacgatatgagc

SEQ ID NO: 90 - DNA, 31 bp, Artificial
  primer sequence E339D,rev
gctcatatcgtcatcatcaccgccccaaccc

SEQ ID NO: 91 - DNA, 32 bp, Artificial
  primer sequence I311Y,fwd
gccgtacgaagattatttcggcggtgtctcag

SEQ ID NO: 92 - DNA, 32 bp, Artificial
  primer sequence I311Y,rev
ctgagacaccgccgaaataatcttcgtacggc